European Patent Application EP 4 417 625 A1, published August 21, 2024. Title: ＭｅｒＴＫに特異的に結合する抗体又はその断片、及び抗腫瘍剤. Applicant: 株式会社カイオム・バイオサイエンス. The sequence listing filed with the application follows.

SEQUENCE LISTING (24 sequences)

SEQ ID NO: 1 - protein, 120 aa, synthetic construct
QVQLQQPGTELVKPGASVKLSCRASGNTFTSYWMHWVKQRPGQGLEWIGNINPSNGGTNYNEKFKSKATLTVDKSSSTAYMQLSSLTSEDSAVYYCARLNYYGFDGFAFWGQGTLVTVSA

SEQ ID NO: 2 - protein, 5 aa, synthetic construct
SYWMH

SEQ ID NO: 3 - protein, 17 aa, synthetic construct
NINPSNGGTNYNEKFKS

SEQ ID NO: 4 - protein, 11 aa, synthetic construct
LNYYGFDGFAF

SEQ ID NO: 5 - protein, 107 aa, synthetic construct
DIKMTQSPSSMYASLGERVTITCKASQDINSYLSWFQQKPGKSPKTLIYRANRLVDGVPSRFSGSGSGQDYSLTISSLEYEDMGIYYCLQYDEFPFTFGSGTKLEIK

SEQ ID NO: 6 - protein, 11 aa, synthetic construct
KASQDINSYLS

SEQ ID NO: 7 - protein, 7 aa, synthetic construct
RANRLVD

SEQ ID NO: 8 - protein, 9 aa, synthetic construct
LQYDEFPFT

SEQ ID NO: 9 - protein, 122 aa, synthetic construct
EVQLVESGGGLVQPKGSLKLSCAASGFTFNVYDMHWVRQAPGEGLEWVARIRSKSSNYATNYADSVKDRFTISRDDSQSMLYLQMNNLQTEDTAIYYCVRDGSHYYYALDYWGQGTSVTVSS

SEQ ID NO: 10 - protein, 5 aa, synthetic construct
VYDMH

SEQ ID NO: 11 - protein, 19 aa, synthetic construct
RIRSKSSNYATNYADSVKD

SEQ ID NO: 12 - protein, 11 aa, synthetic construct
DGSHYYYALDY

SEQ ID NO: 13 - protein, 107 aa, synthetic construct
DIQMTQTTSSLSASLGDRVTISCRASQDINNYLNWYQQKLDGTVKLLIYYSSRLHSGVPSRFSGSGSGTDYSLTISNLEQEDIATYFCQQGKMFPWTFGGGTKLEIK

SEQ ID NO: 14 - protein, 11 aa, synthetic construct
RASQDINNYLN

SEQ ID NO: 15 - protein, 7 aa, synthetic construct
YSSRLHS

SEQ ID NO: 16 - protein, 9 aa, synthetic construct
QQGKMFPWT

SEQ ID NO: 17 - protein, 120 aa, synthetic construct
QVQLQQPGTELVKPGASVKLSCRASGNTFTSYWMHWVKQRPGQGLEWIGNINPSSGGTNYNEKFKSKATLTVDKSSSTAYMQLSSLTSEDSAVYYCARLNYYGFDGFAFWGQGTLVTVSA

SEQ ID NO: 18 - protein, 17 aa, synthetic construct
NINPSSGGTNYNEKFKS

SEQ ID NO: 19 - protein, 107 aa, synthetic construct
DIKMTQSPSSMYASLGERVTITCKASQDINSYLSWFQQKPGKSPKTLIYRANRLVSGVPSRFSGSGSGQDYSLTISSLEYEDMGIYYCLQYDEFPFTFGSGTKLEIK

SEQ ID NO: 20 - protein, 7 aa, synthetic construct
RANRLVS

SEQ ID NO: 21 - protein, 120 aa, synthetic construct
QVQLVQSGAEVKKPGSSVKVSCKASGNTFTSYWMHWVRQAPGQGLEWIGNINPSSGGTNYNEKFKSRVTITVDKSTSTAYMELSSLRSEDTAVYYCARLNYYGFDGFAFWGQGTLVTVSS

SEQ ID NO: 22 - protein, 107 aa, synthetic construct
DIQMTQSPSSLSASVGDRVTITCKASQDINSYLSWFQQKPGKAPKTLIYRANRLVSGVPSRFSGSGSGTDYTLTISSLQPEDFATYYCLQYDEFPFTFGGGTKVEIK

SEQ ID NO: 23 - protein, 122 aa, synthetic construct
EVQLVESGGGLVQPGGSLRLSCAASGFTFNVYDMHWVRQAPGKGLEWVARIRSKSSNYATNYADSVKDRFTISRDDAKNSLYLQMNSLRAEDTAVYYCVRDGSHYYYALDYWGQGTTVTVSS

SEQ ID NO: 24 - protein, 107 aa, synthetic construct
DIQMTQSPSSLSASVGDRVTITCRASQDINNYLNWYQQKPGKAPKLLIYYSSRLHSGVPSRFSGSGSGTDYTLTISSLQPEDFATYYCQQGKMFPWTFGGGTKVEIK